European Patent Application EP 4 635 981 A1, published October 22, 2025. Title: 抗CLL1单域抗体及其应用. Applicant: 浙江康佰裕生物科技有限公司. Application CN. The sequence listing filed with the application follows.

SEQUENCE LISTING (4 sequences)

SEQ ID NO: 1 - protein, 129 aa, synthetic construct
DVQLQESGGGLVQPGGSLRLSCAASGFTFGSYDMTWVRQAPGKGPEWVSGINSGGSSTYYADSVKGRFTISRDNAKNTLYLQMNSLKPEDTAVYYCATIDRLSTVVAGTYQPSEEYDYWGQGTQVTVSS

SEQ ID NO: 2 - DNA, 387 bp, synthetic construct
  source 1..387: mol_type = other DNA
gatgtgcagctgcaggagtctggaggaggcttggtgcagcctgggggttctctgagactctcctgtgcagcctctggattcaccttcggaagctatgacatgacctgggtccgccaggctccaggaaaggggcccgagtgggtctcaggaattaatagtggtggtagtagcacatactatgcagactccgtgaagggccgattcaccatctccagagacaacgccaagaacacgctgtatctgcaaatgaacagcctgaaacctgaggacacggccgtgtattactgtgcaactatcgaccgccttagtacggtagtagctggtacgtaccagccgtccgaagaatatgactactggggccaggggacccaggtcaccgtctccagc

SEQ ID NO: 3 - DNA, 696 bp, Homo sapiens
  source 1..696: mol_type = genomic DNA
gagcccaaatctgctgacaaaactcacacatgcccaccgtgcccagcacctgaactcctggggggaccgtcagtcttcctcttccccccaaaacccaaggacaccctcatgatctcccggacccccgaggtcacatgcgtggtggtggacgtgagccacgaagaccctgaggtcaagttcaactggtacgtggacggcgtggaggtgcataatgccaagacaaagccgcgggaggagcagtacaacagcacgtaccgtgtggtcagcgtcctcaccgtcctgcaccaggactggctgaatggcaaggagtacaagtgcaaggtctccaacaaagccctcccagcccccatcgagaaaaccatctccaaagccaaagggcagccccgagaaccacaggtgtacaccctgcccccatcccgggaggagatgaccaagaaccaggtcagcctgacctgcctggtcaaaggcttctatcccagcgacatcgccgtggagtgggagagcaatgggcagccggagaacaactacaagaccacgcctcccgtgctggactccgacggctccttcttcctctacagcaagctcaccgtggacaagagcaggtggcagcaggggaacgtcttctcatgctccgtgatgcatgaggctctgcacaaccactacacgcagaagagcctctccctgtctccgggtaaa

SEQ ID NO: 4 - protein, 232 aa, Homo sapiens
EPKSADKTHTCPPCPAPELLGGPSVFLFPPKPKDTLMISRTPEVTCVVVDVSHEDPEVKFNWYVDGVEVHNAKTKPREEQYNSTYRVVSVLTVLHQDWLNGKEYKCKVSNKALPAPIEKTISKAKGQPREPQVYTLPPSREEMTKNQVSLTCLVKGFYPSDIAVEWESNGQPENNYKTTPPVLDSDGSFFLYSKLTVDKSRWQQGNVFSCSVMHEALHNHYTQKSLSLSPGK